European Patent Specification EP 3 331 548 B1, published April 15, 2026. Title: ANTI-CD154 ANTIBODY HAVING IMPROVED BINDING, FUNCTIONAL AND SAFETY CHARACTERISTICS AND USE IN HUMAN IMMUNOTHERAPY. Applicant: ROTHSTEIN, Jay. Application TBA. The sequence listing filed with the application follows.

SEQUENCE LISTING (32 sequences)

SEQ ID NO: 1 - protein, 120 aa, Artificial Sequence
  INX021 Variable Heavy
EVQLQESGPGLVKPSETLSLTCTVSGDSITNGFWIWIRKPPGNKLEYMGYISYSGSTYYNPSLKSRISISRDTSKNQFSLKLSSVTAADTGVYYCAYRSYGRTPYYFDYWGQGTTLTVSS

SEQ ID NO: 2 - protein, 107 aa, Artificial Sequence
  INX021 Variable Light
DIVMTQSPSFLSASVGDRVTITCKASSNLGHAVAWYQQKPGKSPKLLIYSASNRYTGVPDRFSGSGSGTDFTLTISSLQPEDFADYFCQQYDDYPYTFGGGTKLEIK

SEQ ID NO: 3 - protein, 330 aa, Artificial Sequence
  INX021 Constant Heavy
ASTKGPSVFPLAPSSKSTSGGTAALGCLVKDYFPEPVTVSWNSGALTSGVHTFPAVLQSSGLYSLSSVVTVPSSSLGTQTYICNVNHKPSNTKVDKKAEPKSCDKTHTCPPCPAPELLGGPSVFLFPPKPKDTLMISRTPEVTCVVVDVSHRDPEVKFNWYVDGVEVHNAKTKPREEQYNSTYRVVSVLTVLHQDWLNGKEYKCAVSNKALPAPIEKTISKAKGQPREPQVYTLPPSRDELTKNQVSLTCLVKGFYPSDIAVEWESNGQPENNYKTTPPVLDSDGSFFLYSKLTVDKSRWQQGNVFSCSVMHEALHNHYTQKSLSLSPGK

SEQ ID NO: 4 - protein, 107 aa, Artificial Sequence [sequence omitted]

SEQ ID NO: 5 - protein, 10 aa, Mus musculus
GDSITNGFWI

SEQ ID NO: 6 - protein, 9 aa, Mus musculus
YISYSGSTY

SEQ ID NO: 7 - protein, 13 aa, Mus musculus
YRSYGRTPYYFDY

SEQ ID NO: 8 - protein, 11 aa, Mus musculus
KASSNLGHAVA

SEQ ID NO: 9 - protein, 7 aa, Mus musculus
SASNRYT

SEQ ID NO: 10 - protein, 9 aa, Mus musculus
QQYDDYPYT

SEQ ID NO: 11 - protein, 330 aa, Homo sapiens [sequence omitted]

SEQ ID NO: 12 - protein, 330 aa, Artificial Sequence [sequence omitted]

SEQ ID NO: 13 - protein, 330 aa, Mus musculus; identical to SEQ ID NO: 3

SEQ ID NO: 14 - protein, 330 aa, Artificial Sequence [sequence omitted]

SEQ ID NO: 15 - protein, 120 aa, Artificial Sequence
  IDEC-131 Variable Heavy-Chain Sequence
EVQLQESGPGLVKPSETLSLTCTVSGDSITNGFWIWIRKPPGNKLEYMGYISYSGSTYYNPSLKSRISISRDTSKNQFSLKLSSVTAADTGVYYCACRSYGRTPYYFDFWGQGTTLTVSS

SEQ ID NO: 16 - protein, 120 aa, Mus musculus
EVQLQESGPGLVKPSETLSLTCTVSGDSITNGFWIWIRKPPGNKLEYMGYISYSGSTYYNPSLKSRISISRDTSKNQFSLKLSSVTAADTGVYYCAYRSYGRTPYYFDFWGQGTTLTVSS

SEQ ID NO: 17 - protein, 120 aa, Homo sapiens; identical to SEQ ID NO: 1

SEQ ID NO: 18 - protein, 120 aa, Artificial Sequence; identical to SEQ ID NO: 16
  Variable heavy-chain sequence consensus

SEQ ID NO: 19 - protein, 107 aa, Mus musculus
DIVMTQSPSFLSASVGDRVTITCKASQNVITAVAWYQQKPGKSPKLLIYSASNRYTGVPDRFSGSGSGTDFTLTISSLQPEDFADYFCQQYDDYPYTFGGGTKLEIK

SEQ ID NO: 20 - protein, 107 aa, Artificial Sequence
  IDEC_AB2-IMX variable light chain sequence
DIVMTQSPSFLSASVGDRVTITCKASQNVITAVAWYQQKPGKSPKLLIYSASNRYTGVPDRFSGSGSGTDFTLTISSLQPEDFADYFCQQYNSYPYTFGGGTKLEIK

SEQ ID NO: 21 - protein, 107 aa, Artificial Sequence
  Variable light-chain sequence 30
DIVMTQSPSFLSASVGDRVTITCKAGHSLGTAVAWYQQKPGKSPKLLIYSASNRYTGVPDRFSGSGSGTDFTLTISSLQPEDFADYFCQQYDDYPYTFGGGTKLEIK

SEQ ID NO: 22 - protein, 107 aa, Artificial Sequence
  Variable light-chain sequence 25
DIVMTQSPSFLSASVGDRVTITCKASQNLNHAVAWYQQKPGKSPKLLIYSASNRYTGVPDRFSGSGSGTDFTLTISSLQPEDFADYFCQQYDDYPYTFGGGTKLEIK

SEQ ID NO: 23 - protein, 107 aa, Artificial Sequence
  Variable light-chain sequence 22
DIVMTQSPSFLSASVGDRVTITCKASSNLGNAVAWYQQKPGKSPKLLIYSASNRYTGVPDRFSGSGSGTDFTLTISSLQPEDFADYFCQQYDDYPYTFGGGTKLEIK

SEQ ID NO: 24 - protein, 107 aa, Artificial Sequence; identical to SEQ ID NO: 2
  Variable light-chain sequence 21

SEQ ID NO: 25 - protein, 107 aa, Artificial Sequence
  Variable light-chain sequence 28
DIVMTQSPSFLSASVGDRVTITCKAPSSLGHAVAWYQQKPGKSPKLLIYSASNRYTGVPDRFSGSGSGTDFTLTISSLQPEDFADYFCQQYDDYPYTFGGGTKLEIK

SEQ ID NO: 26 - protein, 107 aa, Artificial Sequence
  Variable light-chain sequence 23
DIVMTQSPSFLSASVGDRVTITCKGSSPLGHAVAWYQQKPGKSPKLLIYSASNRYTGVPDRFSGSGSGTDFTLTISSLQPEDFADYFCQQYDDYPYTFGGGTKLEIK

SEQ ID NO: 27 - protein, 107 aa, Artificial sequence
  Variable light-chain sequence 31
DIVMTQSPSFLSASVGDRVTITCKANQPLGHAVAWYQQKPGKSPKLLIYSASNRYTGVPDRFSGSGSGTDFTLTISSLQPEDFADYFCQQYDDYPYTFGGGTKLEIK

SEQ ID NO: 28 - protein, 107 aa, Artificial Sequence
  Variable light-chain sequence 29
DIVMTQSPSFLSASVGDRVTITCKGNQPLGHAVAWYQQKPGKSPKLLIYSASNRYTGVPDRFSGSGSGTDFTLTISSLQPEDFADYFCQQYDDYPYTFGGGTKLEIK

SEQ ID NO: 29 - protein, 107 aa, Artificial Sequence
  Variable light-chain sequence 27
DIVMTQSPSFLSASVGDRVTITCKASQHLGHAVAWYQQKPGKSPKLLIYSASNRYTGVPDRFSGSGSGTDFTLTISSLQPEDFADYFCQQYDDYPYTFGGGTKLEIK

SEQ ID NO: 30 - protein, 107 aa, Artificial Sequence
  Variable light-chain sequence 26
DIVMTQSPSFLSASVGDRVTITCKASQHLGTAVAWYQQKPGKSPKLLIYSASNRYTGVPDRFSGSGSGTDFTLTISSLQPEDFADYFCQQYDDYPYTFGGGTKLEIK

SEQ ID NO: 31 - protein, 107 aa, Artificial Sequence
  Variable light-chain sequence 24
DIVMTQSPSFLSASVGDRVTITCKAPQNLGTAVAWYQQKPGKSPKLLIYSASNRYTGVPDRFSGSGSGTDFTLTISSLQPEDFADYFCQQYDDYPYTFGGGTKLEIK

SEQ ID NO: 32 - protein, 107 aa, Artificial Sequence
  Variable light-chain sequence consensus
DIVMTQSPSFLSASVGDRVTITCKASQNLGHAVAWYQQKPGKSPKLLIYSASNRYTGVPDRFSGSGSGTDFTLTISSLQPEDFADYFCQQYDDYPYTFGGGTKLEIK